European Patent Application EP 4 299 592 A1, published January 3, 2024. Title: T cell co-expressing CXCR2 and a STAR against GPC3 and uses thereof. Applicant: CHINA IMMUNOTECH (BEIJING) BIOTECHNOLOGY CO., LTD. The sequence listing filed with the application follows.

SEQUENCE LISTING (34 sequences)

SEQ ID NO: 1 - protein, 141 aa, Homo sapiens
DIQNPDPAVYQLRDSKSSDKSVCLFTDFDSQTNVSQSKDSDVYITDKTVLDMRSMDFKSNSAVAWSNKSDFACANAFNNSIIPEDTFFPSPESSCDVKLVEKSFETDTNLNFQNLSVIGFRILLLKVAGFNLLMTLRLWSS

SEQ ID NO: 2 - protein, 137 aa, Mus musculus
DIQNPEPAVYQLKDPRSQDSTLCLFTDFDSQINVPKTMESGTFITDKTVLDMKAMDSKSNGAIAWSNQTSFTCQDIFKETNATYPSSDVPCDATLTEKSFETDMNLNFQNLSVMGLRILLLKVAGFNLLMTLRLWSS

SEQ ID NO: 3 - protein, 137 aa, artificial sequence
  mouse T cell receptor alpha chain constant region containing cysteine substitution and modification of hydrophobic region (TRAC-Cys-TM)
DIQNPEPAVYQLKDPRSQDSTLCLFTDFDSQINVPKTMESGTFITDKCVLDMKAMDSKSNGAIAWSNQTSFTCQDIFKETNATYPSSDVPCDATLTEKSFETDMNLNFQNLLVIVLRILLLKVAGFNLLMTLRLWSS

SEQ ID NO: 4 - protein, 133 aa, artificial sequence
  mouse T cell receptor alpha chain constant region containing N-terminal modification, cysteine substitution and modification of transmembrane hydrophobic region (TRAC-Nrec-Cys-TM)
DIQNPDPAVYQLRDDSTLCLFTDFDSQINVPKTMESGTFITDKCVLDMKAMDSKSNGAIAWSNQTSFTCQDIFKETNATYPSSDVPCDATLTEKSFETDMNLNFQNLLVIVLRILLLKVAGFNLLMTLRLWSS

SEQ ID NO: 5 - protein, 176 aa, Homo sapiens
DLKNVFPPEVAVFEPSEAEISHTQKATLVCLATGFYPDHVELSWWVNGKEVHSGVSTDPQPLKEQPALNDSRYCLSSRLRVSATFWQNPRNHFRCQVQFYGLSENDEWTQDRAKPVTQIVSAEAWGRADCGFTSESYQQGVLSATILYEILLGKATLYAVLVSALVLMAMVKRKDF

SEQ ID NO: 6 - protein, 172 aa, Mus musculus
DLRNVTPPKVSLFEPSKAEIANKQKATLVCLARGFFPDHVELSWWVNGKEVHSGVSTDPQAYKESNYSYCLSSRLRVSATFWHNPRNHFRCQVQFHGLSEEDKWPEGSPKPVTQNISAEAWGRADCGITSASYQQGVLSATILYEILLGKATLYAVLVSTLVVMAMVKRKNS

SEQ ID NO: 7 - protein, 172 aa, artificial sequence
  mouse T cell receptor beta chain constant region containing cysteine substitution (TRBC-Cys-TM)
DLRNVTPPKVSLFEPSKAEIANKQKATLVCLARGFFPDHVELSWWVNGKEVHSGVCTDPQAYKESNYSYCLSSRLRVSATFWHNPRNHFRCQVQFHGLSEEDKWPEGSPKPVTQNISAEAWGRADCGITSASYQQGVLSATILYEILLGKATLYAVLVSTLVVMAMVKRKNS

SEQ ID NO: 8 - protein, 166 aa, artificial sequence
  mouse T cell receptor beta chain constant region containing N-terminal modification, and cysteine substitution (TRBC-Nrecc-Cys-TM)
DLKNVFPPEVAVFEPSAEIATLVCLARGFFPDHVELSWWVNGKEVHSGVCTDPQAYKESNYSYCLSSRLRVSATFWHNPRNHFRCQVQFHGLSEEDKWPEGSPKPVTQNISAEAWGRADCGITSASYQQGVLSATILYEILLGKATLYAVLVSTLVVMAMVKRKNS

SEQ ID NO: 9 - protein, 115 aa, artificial sequence
  Anti-GPC3 GC33 VH
QVQLVQSGAEVKKPGASVKVSCKASGYTFTDYEMHWVRQAPGQGLEWMGALDPKTGDTAYSQKFKGRVTLTADESTSTAYMELSSLRSEDTAVYYCTRFYSYTYWGQGTLVTVSS

SEQ ID NO: 10 - protein, 113 aa, artificial sequence
  Anti-GPC3 GC33 VL
DVVMTQSPLSLPVTPGEPASISCRSSQSLVHSNRNTYLHWYLQKPGQSPQLLIYKVSNRFSGVPDRFSGSGSGTDFTLKISRVEAEDVGVYYCSQNTHVPPTFGQGTKLEIKR

SEQ ID NO: 11 - protein, 37 aa, artificial sequence
  OX40 endodomain
RRDQRLPPDAHKPPGGGSFRTPIQEEQADAHSTLAKI

SEQ ID NO: 12 - protein, 360 aa, artificial sequence
  CXCR2 amino acid sequence
MEDFNMESDSFEDFWKGEDLSNYSYSSTLPPFLLDAAPCEPESLEINKYFVVIIYALVFLLSLLGNSLVMLVILYSRVGRSVTDVYLLNLALADLLFALTLPIWAASKVNGWIFGTFLCKVVSLLKEVNFYSGILLLACISVDRYLAIVHATRTLTQKRYLVKFICLSIWGLSLLLALPVLLFRRTVYSSNVSPACYEDMGNNTANWRMLLRILPQSFGFIVPLLIMLFCYGFTLRTLFKAHMGQKHRAMRVIFAVVLIFLLCWLPYNLVLLADTLMRTQVIQETCERRNHIDRALDATEILGILHSCLNPLIYAFIGQKFRHGLLKILAIHGLISKDSLPKDSRPSFVGSSSGHTSTTL

SEQ ID NO: 13 - protein, 252 aa, artificial sequence
  GPC3 STAR-CXCR2(TRAC-Cys-TM) alpha chain
QVQLVQSGAEVKKPGASVKVSCKASGYTFTDYEMHWVRQAPGQGLEWMGALDPKTGDTAYSQKFKGRVTLTADESTSTAYMELSSLRSEDTAVYYCTRFYSYTYWGQGTLVTVSSDIQNPEPAVYQLKDPRSQDSTLCLFTDFDSQINVPKTMESGTFITDKCVLDMKAMDSKSNGAIAWSNQTSFTCQDIFKETNATYPSSDVPCDATLTEKSFETDMNLNFQNLLVIVLRILLLKVAGFNLLMTLRLWSS

SEQ ID NO: 14 - protein, 286 aa, artificial sequence
  GPC3 STAR-CXCR2(TRBC-Cys-TM) beta chain
DVVMTQSPLSLPVTPGEPASISCRSSQSLVHSNRNTYLHWYLQKPGQSPQLLIYKVSNRFSGVPDRFSGSGSGTDFTLKISRVEAEDVGVYYCSQNTHVPPTFGQGTKLEIKREDLRNVTPPKVSLFEPSKAEIANKQKATLVCLARGFFPDHVELSWWVNGKEVHSGVCTDPQAYKESNYSYCLSSRLRVSATFWHNPRNHFRCQVQFHGLSEEDKWPEGSPKPVTQNISAEAWGRADCGITSASYQQGVLSATILYEILLGKATLYAVLVSTLVVMAMVKRKNS

SEQ ID NO: 15 - protein, 302 aa, artificial sequence
  GPC3 STAR-OX40-CXCR2 (TRAC-Cys-TM) alpha chain
QVQLVQSGAEVKKPGASVKVSCKASGYTFTDYEMHWVRQAPGQGLEWMGALDPKTGDTAYSQKFKGRVTLTADESTSTAYMELSSLRSEDTAVYYCTRFYSYTYWGQGTLVTVSSDIQNPEPAVYQLKDPRSQDSTLCLFTDFDSQINVPKTMESGTFITDKCVLDMKAMDSKSNGAIAWSNQTSFTCQDIFKETNATYPSSDVPCDATLTEKSFETDMNLNFQNLLVIVLRILLLKVAGFNLLMTLRLWGGGGSGGGGSGGGGSRRDQRLPPDAHKPPGGGSFRTPIQEEQADAHSTLAKI

SEQ ID NO: 16 - protein, 302 aa, artificial sequence; identical to SEQ ID NO: 15
  GPC3 STAR-OX40-CXCR2(TCRbC-Cys-TM) beta chain

SEQ ID NO: 17 - protein, 248 aa, artificial sequence
  GPC3 STAR-CXCR2(TRAC-Nrec-Cys-TM) alpha chain
QVQLVQSGAEVKKPGASVKVSCKASGYTFTDYEMHWVRQAPGQGLEWMGALDPKTGDTAYSQKFKGRVTLTADESTSTAYMELSSLRSEDTAVYYCTRFYSYTYWGQGTLVTVSSDIQNPDPAVYQLRDDSTLCLFTDFDSQINVPKTMESGTFITDKCVLDMKAMDSKSNGAIAWSNQTSFTCQDIFKETNATYPSSDVPCDATLTEKSFETDMNLNFQNLLVIVLRILLLKVAGFNLLMTLRLWSS

SEQ ID NO: 18 - protein, 279 aa, artificial sequence
  GPC3 STAR-CXCR2(TRBC- Nrec-Cys-TM) beta chain
DVVMTQSPLSLPVTPGEPASISCRSSQSLVHSNRNTYLHWYLQKPGQSPQLLIYKVSNRFSGVPDRFSGSGSGTDFTLKISRVEAEDVGVYYCSQNTHVPPTFGQGTKLEIKRDLKNVFPPEVAVFEPSAEIATLVCLARGFFPDHVELSWWVNGKEVHSGVCTDPQAYKESNYSYCLSSRLRVSATFWHNPRNHFRCQVQFHGLSEEDKWPEGSPKPVTQNISAEAWGRADCGITSASYQQGVLSATILYEILLGKATLYAVLVSTLVVMAMVKRKNS

SEQ ID NO: 19 - protein, 298 aa, artificial sequence
  GPC3 STAR-OX40-CXCR2 (TRAC- Nrec-Cys-TM) alpha chain
QVQLVQSGAEVKKPGASVKVSCKASGYTFTDYEMHWVRQAPGQGLEWMGALDPKTGDTAYSQKFKGRVTLTADESTSTAYMELSSLRSEDTAVYYCTRFYSYTYWGQGTLVTVSSDIQNPDPAVYQLRDDSTLCLFTDFDSQINVPKTMESGTFITDKCVLDMKAMDSKSNGAIAWSNQTSFTCQDIFKETNATYPSSDVPCDATLTEKSFETDMNLNFQNLLVIVLRILLLKVAGFNLLMTLRLWGGGGSGGGGSGGGGSRRDQRLPPDAHKPPGGGSFRTPIQEEQADAHSTLAKI

SEQ ID NO: 20 - protein, 325 aa, artificial sequence
  GPC3 STAR-OX40-CXCR2(TRBC- Nrec-Cys-TM) beta chain
DVVMTQSPLSLPVTPGEPASISCRSSQSLVHSNRNTYLHWYLQKPGQSPQLLIYKVSNRFSGVPDRFSGSGSGTDFTLKISRVEAEDVGVYYCSQNTHVPPTFGQGTKLEIKRDLKNVFPPEVAVFEPSAEIATLVCLARGFFPDHVELSWWVNGKEVHSGVCTDPQAYKESNYSYCLSSRLRVSATFWHNPRNHFRCQVQFHGLSEEDKWPEGSPKPVTQNISAEAWGRADCGITSASYQQGVLSATILYEILLGKATLYAVLVSTLVVMAMGGGGSGGGGSGGGGSRRDQRLPPDAHKPPGGGSFRTPIQEEQADAHSTLAKI

SEQ ID NO: 21 - protein, 477 aa, artificial sequence
  GPC3 CAR-CXCR2
DVVMTQSPLSLPVTPGEPASISCRSSQSLVHSNRNTYLHWYLQKPGQSPQLLIYKVSNRFSGVPDRFSGSGSGTDFTLKISRVEAEDVGVYYCSQNTHVPPTFGQGTKLEIKRGGGGSGGGGSGGGGSQVQLVQSGAEVKKPGASVKVSCKASGYTFTDYEMHWVRQAPGQGLEWMGALDPKTGDTAYSQKFKGRVTLTADESTSTAYMELSSLRSEDTAVYYCTRFYSYTYWGQGTLVTVSSSRSHFVPVFLPAKPTTTPAPRPPTPAPTIASQPLSLRPEACRPAAGGAVHTRGLDFACDIYIWAPLAGTCGVLLLSLVITKRGRKKLLYIFKQPFMRPVQTTQEEDGCSCRFPEEEEGGCELRVKFSRSADAPAYQQGQNQLYNELNLGRREEYDVLDKRRGRDPEMGGKPRRKNPQEGLYNELQKDKMAEAYSEIGMKGERRRGKGHDGLYQGLSTATKDTYDALHMQALPPR

SEQ ID NO: 22 - protein, 8 aa, artificial sequence
  heavy chain variable region CDR1 amino acid sequence
GYTFTDYE

SEQ ID NO: 23 - protein, 8 aa, artificial sequence
  heavy chain variable region CDR2 amino acid sequence
LDPKTGDT

SEQ ID NO: 24 - protein, 2 aa, artificial sequence
  heavy chain variable region CDR3 amino acid sequence
TR

SEQ ID NO: 25 - protein, 11 aa, artificial sequence
  light chain variable region CDR1 amino acid sequence
QSLVHSNRNTY

SEQ ID NO: 26 - protein, 3 aa, artificial sequence
  light chain variable region CDR2 amino acid sequence
KVS

SEQ ID NO: 27 - protein, 7 aa, artificial sequence
  light chain variable region CDR3 amino acid sequence
SQNTHVP

SEQ ID NO: 28 - protein, 135 aa, artificial sequence
  Endodomain-deleted mouse T cell receptor alpha chain constant region
DIQNPEPAVYQLKDPRSQDSTLCLFTDFDSQINVPKTMESGTFITDKTVLDMKAMDSKSNGAIAWSNQTSFTCQDIFKETNATYPSSDVPCDATLTEKSFETDMNLNFQNLSVMGLRILLLKVAGFNLLMTLRLW

SEQ ID NO: 29 - protein, 135 aa, artificial sequence
  Endodomain-deleted mouse T cell receptor alpha chain constant region with cysteine substitution and hydrophobic modification
DIQNPEPAVYQLKDPRSQDSTLCLFTDFDSQINVPKTMESGTFITDKCVLDMKAMDSKSNGAIAWSNQTSFTCQDIFKETNATYPSSDVPCDATLTEKSFETDMNLNFQNLLVIVLRILLLKVAGFNLLMTLRLW

SEQ ID NO: 30 - protein, 131 aa, artificial sequence
  Endodomain-deleted mouse T cell receptor alpha chain constant region with N-terminal modification, cysteine substitution and modification of transmembrane hydrophobic region
DIQNPDPAVYQLRDDSTLCLFTDFDSQINVPKTMESGTFITDKCVLDMKAMDSKSNGAIAWSNQTSFTCQDIFKETNATYPSSDVPCDATLTEKSFETDMNLNFQNLLVIVLRILLLKVAGFNLLMTLRLW

SEQ ID NO: 31 - protein, 166 aa, artificial sequence
  Endodomain-deleted mouse T cell receptor beta chain constant region
DLRNVTPPKVSLFEPSKAEIANKQKATLVCLARGFFPDHVELSWWVNGKEVHSGVSTDPQAYKESNYSYCLSSRLRVSATFWHNPRNHFRCQVQFHGLSEEDKWPEGSPKPVTQNISAEAWGRADCGITSASYQQGVLSATILYEILLGKATLYAVLVSTLVVMAM

SEQ ID NO: 32 - protein, 166 aa, artificial sequence
  Endodomain-deleted mouse T cell receptor beta chain constant region with cysteine substitution
DLRNVTPPKVSLFEPSKAEIANKQKATLVCLARGFFPDHVELSWWVNGKEVHSGVCTDPQAYKESNYSYCLSSRLRVSATFWHNPRNHFRCQVQFHGLSEEDKWPEGSPKPVTQNISAEAWGRADCGITSASYQQGVLSATILYEILLGKATLYAVLVSTLVVMAM

SEQ ID NO: 33 - protein, 160 aa, artificial sequence
  Endodomain-deleted mouse T cell receptor beta chain constant region with N-terminal modification and cysteine substitution
DLKNVFPPEVAVFEPSAEIATLVCLARGFFPDHVELSWWVNGKEVHSGVCTDPQAYKESNYSYCLSSRLRVSATFWHNPRNHFRCQVQFHGLSEEDKWPEGSPKPVTQNISAEAWGRADCGITSASYQQGVLSATILYEILLGKATLYAVLVSTLVVMAM

SEQ ID NO: 34 - protein, 15 aa, artificial sequence
  (G4S)3 linker
GGGGSGGGGSGGGGS